European Patent Specification EP 4 043 556 B1, published February 7, 2024. Title: METHODS FOR IMPROVING FUNCTIONALITY IN NK CELL BY GENE INACTIVATION USING SPECIFIC ENDONUCLEASE. Applicant: CELLECTIS. The sequence listing filed with the application follows.

SEQUENCE LISTING (30 sequences)

SEQ ID NO: 1 - DNA, 49 bp, homo sapiens
  TGF-B Exon 2 target
ttgagctggacaccctggtggggaaaggtcgctttgctgaggtctataa

SEQ ID NO: 2 - protein, 936 aa, artificial sequence
  Left Talen for TGF-B Exon 2 target
MGDPKKKRKVIDYPYDVPDYAIDIADLRTLGYSQQQQEKIKPKVRSTVAQHHEALVGHGFTHAHIVALSQHPAALGTVAVKYQDMIAALPEATHEAIVGVGKQWSGARALEALLTVAGELRGPPLQLDTGQLLKIAKRGGVTAVEAVHAWRNALTGAPLNLTPQQVVAIASNGGGKQALETVQRLLPVLCQAHGLTPQQVVAIASNNGGKQALETVQRLLPVLCQAHGLTPEQVVAIASNIGGKQALETVQALLPVLCQAHGLTPQQVVAIASNNGGKQALETVQRLLPVLCQAHGLTPEQVVAIASHDGGKQALETVQRLLPVLCQAHGLTPQQVVAIASNGGGKQALETVQRLLPVLCQAHGLTPQQVVAIASNNGGKQALETVQRLLPVLCQAHGLTPQQVVAIASNNGGKQALETVQRLLPVLCQAHGLTPEQVVAIASNIGGKQALETVQALLPVLCQAHGLTPEQVVAIASHDGGKQALETVQRLLPVLCQAHGLTPEQVVAIASNIGGKQALETVQALLPVLCQAHGLTPEQVVAIASHDGGKQALETVQRLLPVLCQAHGLTPEQVVAIASHDGGKQALETVQRLLPVLCQAHGLTPEQVVAIASHDGGKQALETVQRLLPVLCQAHGLTPQQVVAIASNGGGKQALETVQRLLPVLCQAHGLTPQQVVAIASNGGGRPALESIVAQLSRPDPALAALTNDHLVALACLGGRPALDAVKKGLGDPISRSQLVKSELEEKKSELRHKLKYVPHEYIELIEIARNSTQDRILEMKVMEFFMKVYGYRGKHLGGSRKPDGAIYTVGSPIDYGVIVDTKAYSGGYNLPIGQADEMQRYVEENQTRNKHINPNEWWKVYPSSVTEFKFLFVSGHFKGNYKAQLTRLNHITNCNGAVLSVEELLIGGEMIKAGTLTLEEVRRKFNNGEINFAAD

SEQ ID NO: 3 - protein, 936 aa, artificial sequence
  Right Talen for TGF-B Exon 2 target
MGDPKKKRKVIDYPYDVPDYAIDIADLRTLGYSQQQQEKIKPKVRSTVAQHHEALVGHGFTHAHIVALSQHPAALGTVAVKYQDMIAALPEATHEAIVGVGKQWSGARALEALLTVAGELRGPPLQLDTGQLLKIAKRGGVTAVEAVHAWRNALTGAPLNLTPQQVVAIASNGGGKQALETVQRLLPVLCQAHGLTPEQVVAIASNIGGKQALETVQALLPVLCQAHGLTPQQVVAIASNGGGKQALETVQRLLPVLCQAHGLTPEQVVAIASNIGGKQALETVQALLPVLCQAHGLTPQQVVAIASNNGGKQALETVQRLLPVLCQAHGLTPEQVVAIASNIGGKQALETVQALLPVLCQAHGLTPEQVVAIASHDGGKQALETVQRLLPVLCQAHGLTPEQVVAIASHDGGKQALETVQRLLPVLCQAHGLTPQQVVAIASNGGGKQALETVQRLLPVLCQAHGLTPEQVVAIASHDGGKQALETVQRLLPVLCQAHGLTPEQVVAIASNIGGKQALETVQALLPVLCQAHGLTPQQVVAIASNNGGKQALETVQRLLPVLCQAHGLTPEQVVAIASHDGGKQALETVQRLLPVLCQAHGLTPEQVVAIASNIGGKQALETVQALLPVLCQAHGLTPEQVVAIASNIGGKQALETVQALLPVLCQAHGLTPQQVVAIASNGGGRPALESIVAQLSRPDPALAALTNDHLVALACLGGRPALDAVKKGLGDPISRSQLVKSELEEKKSELRHKLKYVPHEYIELIEIARNSTQDRILEMKVMEFFMKVYGYRGKHLGGSRKPDGAIYTVGSPIDYGVIVDTKAYSGGYNLPIGQADEMQRYVEENQTRNKHINPNEWWKVYPSSVTEFKFLFVSGHFKGNYKAQLTRLNHITNCNGAVLSVEELLIGGEMIKAGTLTLEEVRRKFNNGEINFAAD

SEQ ID NO: 4 - DNA, 45 bp, homo sapiens
  Cbl-b Exon 2 target
tgtgccaaaatcccaaacttcagttgaaaaatagcccaccatata

SEQ ID NO: 5 - protein, 1065 aa, artificial sequence
  Left Talen for Cbl-b Exon 2 target
MGDPKKKRKVIDYPYDVPDYAIDIADPIRSRTPSPARELLPGPQPDGVQPTADRGVSPPAGGPLDGLPARRTMSRTRLPSPPAPSPAFSAGSFSDLLRQFDPSLFNTSLFDSLPPFGAHHTEAATGEWDEVQSGLRAADAPPPTMRVAVTAARPPRAKPAPRRRAAQPSDASPAAQVDLRTLGYSQQQQEKIKPKVRSTVAQHHEALVGHGFTHAHIVALSQHPAALGTVAVKYQDMIAALPEATHEAIVGVGKQWSGARALEALLTVAGELRGPPLQLDTGQLLKIAKRGGVTAVEAVHAWRNALTGAPLNLTPQQVVAIASNNGGKQALETVQRLLPVLCQAHGLTPQQVVAIASNGGGKQALETVQRLLPVLCQAHGLTPQQVVAIASNNGGKQALETVQRLLPVLCQAHGLTPEQVVAIASHDGGKQALETVQRLLPVLCQAHGLTPEQVVAIASHDGGKQALETVQRLLPVLCQAHGLTPEQVVAIASNIGGKQALETVQALLPVLCQAHGLTPEQVVAIASNIGGKQALETVQALLPVLCQAHGLTPEQVVAIASNIGGKQALETVQALLPVLCQAHGLTPEQVVAIASNIGGKQALETVQALLPVLCQAHGLTPQQVVAIASNGGGKQALETVQRLLPVLCQAHGLTPEQVVAIASHDGGKQALETVQRLLPVLCQAHGLTPEQVVAIASHDGGKQALETVQRLLPVLCQAHGLTPEQVVAIASHDGGKQALETVQRLLPVLCQAHGLTPEQVVAIASNIGGKQALETVQALLPVLCQAHGLTPEQVVAIASNIGGKQALETVQALLPVLCQAHGLTPQQVVAIASNGGGRPALESIVAQLSRPDPSGSGSGGDPISRSQLVKSELEEKKSELRHKLKYVPHEYIELIEIARNSTQDRILEMKVMEFFMKVYGYRGKHLGGSRKPDGAIYTVGSPIDYGVIVDTKAYSGGYNLPIGQADEMQRYVEENQTRNKHINPNEWWKVYPSSVTEFKFLFVSGHFKGNYKAQLTRLNHITNCNGAVLSVEELLIGGEMIKAGTLTLEEVRRKFNNGEINFAAD

SEQ ID NO: 6 - protein, 1065 aa, artificial sequence
  Right Talen for TGF-B Exon 2 target
MGDPKKKRKVIDYPYDVPDYAIDIADPIRSRTPSPARELLPGPQPDGVQPTADRGVSPPAGGPLDGLPARRTMSRTRLPSPPAPSPAFSAGSFSDLLRQFDPSLFNTSLFDSLPPFGAHHTEAATGEWDEVQSGLRAADAPPPTMRVAVTAARPPRAKPAPRRRAAQPSDASPAAQVDLRTLGYSQQQQEKIKPKVRSTVAQHHEALVGHGFTHAHIVALSQHPAALGTVAVKYQDMIAALPEATHEAIVGVGKQWSGARALEALLTVAGELRGPPLQLDTGQLLKIAKRGGVTAVEAVHAWRNALTGAPLNLTPEQVVAIASNIGGKQALETVQALLPVLCQAHGLTPQQVVAIASNGGGKQALETVQRLLPVLCQAHGLTPEQVVAIASNIGGKQALETVQALLPVLCQAHGLTPQQVVAIASNGGGKQALETVQRLLPVLCQAHGLTPQQVVAIASNNGGKQALETVQRLLPVLCQAHGLTPQQVVAIASNNGGKQALETVQRLLPVLCQAHGLTPQQVVAIASNGGGKQALETVQRLLPVLCQAHGLTPQQVVAIASNNGGKQALETVQRLLPVLCQAHGLTPQQVVAIASNNGGKQALETVQRLLPVLCQAHGLTPQQVVAIASNNGGKQALETVQRLLPVLCQAHGLTPEQVVAIASHDGGKQALETVQRLLPVLCQAHGLTPQQVVAIASNGGGKQALETVQRLLPVLCQAHGLTPEQVVAIASNIGGKQALETVQALLPVLCQAHGLTPQQVVAIASNGGGKQALETVQRLLPVLCQAHGLTPQQVVAIASNGGGKQALETVQRLLPVLCQAHGLTPQQVVAIASNGGGRPALESIVAQLSRPDPSGSGSGGDPISRSQLVKSELEEKKSELRHKLKYVPHEYIELIEIARNSTQDRILEMKVMEFFMKVYGYRGKHLGGSRKPDGAIYTVGSPIDYGVIVDTKAYSGGYNLPIGQADEMQRYVEENQTRNKHINPNEWWKVYPSSVTEFKFLFVSGHFKGNYKAQLTRLNHITNCNGAVLSVEELLIGGEMIKAGTLTLEEVRRKFNNGEINFAAD

SEQ ID NO: 7 - DNA, 45 bp, homo sapiens
  Cbl-b Exon 3 target
tgctgctgaattctggagaaagttttttggagacaagtaagtaaa

SEQ ID NO: 8 - protein, 1065 aa, artificial sequence
  Left Talen for Cbl-b Exon 3 target
MGDPKKKRKVIDYPYDVPDYAIDIADPIRSRTPSPARELLPGPQPDGVQPTADRGVSPPAGGPLDGLPARRTMSRTRLPSPPAPSPAFSAGSFSDLLRQFDPSLFNTSLFDSLPPFGAHHTEAATGEWDEVQSGLRAADAPPPTMRVAVTAARPPRAKPAPRRRAAQPSDASPAAQVDLRTLGYSQQQQEKIKPKVRSTVAQHHEALVGHGFTHAHIVALSQHPAALGTVAVKYQDMIAALPEATHEAIVGVGKQWSGARALEALLTVAGELRGPPLQLDTGQLLKIAKRGGVTAVEAVHAWRNALTGAPLNLTPQQVVAIASNNGGKQALETVQRLLPVLCQAHGLTPEQVVAIASHDGGKQALETVQRLLPVLCQAHGLTPQQVVAIASNGGGKQALETVQRLLPVLCQAHGLTPQQVVAIASNNGGKQALETVQRLLPVLCQAHGLTPEQVVAIASHDGGKQALETVQRLLPVLCQAHGLTPQQVVAIASNGGGKQALETVQRLLPVLCQAHGLTPQQVVAIASNNGGKQALETVQRLLPVLCQAHGLTPEQVVAIASNIGGKQALETVQALLPVLCQAHGLTPEQVVAIASNIGGKQALETVQALLPVLCQAHGLTPQQVVAIASNGGGKQALETVQRLLPVLCQAHGLTPQQVVAIASNGGGKQALETVQRLLPVLCQAHGLTPEQVVAIASHDGGKQALETVQRLLPVLCQAHGLTPQQVVAIASNGGGKQALETVQRLLPVLCQAHGLTPQQVVAIASNNGGKQALETVQRLLPVLCQAHGLTPQQVVAIASNNGGKQALETVQRLLPVLCQAHGLTPQQVVAIASNGGGRPALESIVAQLSRPDPSGSGSGGDPISRSQLVKSELEEKKSELRHKLKYVPHEYIELIEIARNSTQDRILEMKVMEFFMKVYGYRGKHLGGSRKPDGAIYTVGSPIDYGVIVDTKAYSGGYNLPIGQADEMQRYVEENQTRNKHINPNEWWKVYPSSVTEFKFLFVSGHFKGNYKAQLTRLNHITNCNGAVLSVEELLIGGEMIKAGTLTLEEVRRKFNNGEINFAAD

SEQ ID NO: 9 - protein, 1065 aa, artificial sequence
  Right Talen for TGF-B Exon 3 target
MGDPKKKRKVIDYPYDVPDYAIDIADPIRSRTPSPARELLPGPQPDGVQPTADRGVSPPAGGPLDGLPARRTMSRTRLPSPPAPSPAFSAGSFSDLLRQFDPSLFNTSLFDSLPPFGAHHTEAATGEWDEVQSGLRAADAPPPTMRVAVTAARPPRAKPAPRRRAAQPSDASPAAQVDLRTLGYSQQQQEKIKPKVRSTVAQHHEALVGHGFTHAHIVALSQHPAALGTVAVKYQDMIAALPEATHEAIVGVGKQWSGARALEALLTVAGELRGPPLQLDTGQLLKIAKRGGVTAVEAVHAWRNALTGAPLNLTPQQVVAIASNGGGKQALETVQRLLPVLCQAHGLTPQQVVAIASNGGGKQALETVQRLLPVLCQAHGLTPEQVVAIASNIGGKQALETVQALLPVLCQAHGLTPEQVVAIASHDGGKQALETVQRLLPVLCQAHGLTPQQVVAIASNGGGKQALETVQRLLPVLCQAHGLTPQQVVAIASNGGGKQALETVQRLLPVLCQAHGLTPEQVVAIASNIGGKQALETVQALLPVLCQAHGLTPEQVVAIASHDGGKQALETVQRLLPVLCQAHGLTPQQVVAIASNGGGKQALETVQRLLPVLCQAHGLTPQQVVAIASNGGGKQALETVQRLLPVLCQAHGLTPQQVVAIASNNGGKQALETVQRLLPVLCQAHGLTPQQVVAIASNGGGKQALETVQRLLPVLCQAHGLTPEQVVAIASHDGGKQALETVQRLLPVLCQAHGLTPQQVVAIASNGGGKQALETVQRLLPVLCQAHGLTPEQVVAIASHDGGKQALETVQRLLPVLCQAHGLTPQQVVAIASNGGGRPALESIVAQLSRPDPSGSGSGGDPISRSQLVKSELEEKKSELRHKLKYVPHEYIELIEIARNSTQDRILEMKVMEFFMKVYGYRGKHLGGSRKPDGAIYTVGSPIDYGVIVDTKAYSGGYNLPIGQADEMQRYVEENQTRNKHINPNEWWKVYPSSVTEFKFLFVSGHFKGNYKAQLTRLNHITNCNGAVLSVEELLIGGEMIKAGTLTLEEVRRKFNNGEINFAAD

SEQ ID NO: 10 - protein, 557 aa, homo sapiens
  CD19 antigen
MPPPRLLFFLLFLTPMEVRPEEPLVVKVEEGDNAVLQCLKGTSDGPTQQLTWSRESPLKPFLKLSLGLPGLGIHMRPLAIWLFIFNVSQQMGGFYLCQPGPPSEKAWQPGWTVNVEGSGELFRWNVSDLGGLGCGLKNRSSEGPSSPSGKLMSPKLYVWAKDRPEIWEGEPPCLPPRDSLNQSLSQDLTMAPGSTLWLSCGVPPDSVSRGPLSWTHVHPKGPKSLLSLELKDDRPARDMWVMETGLLLPRATAQDAGKYYCHRGNLTMSFHLEITARPVLWHWLLRTGGWKVSAVTLAYLIFCLCSLVGILHLQRALVLRRKRKRMTDPTRRFFKVTPPPGSGPQNQYGNVLSLPTPTSGLGRAQRWAAGLGGTAPSYGNPSSDVQADGALGSRSPPGVGPEEEEGEGYEEPDSEEDSEFYENDSNLGQDQLSQDGSGYENPEDEPLGPEDEDSFSNAESYENEDEELTQPVARTMDFLSPHGSAWDPSREATSLAGSQSYEDMRGILYAAPQLRSIRGQPGPNHEEDADSYENMDNPDGPDPAWGGGGRMGTWSTR

SEQ ID NO: 11 - protein, 300 aa, homo sapiens
  CD38 antigen
MANCEFSPVSGDKPCCRLSRRAQLCLGVSILVLILVVVLAVVVPRWRQQWSGPGTTKRFPETVLARCVKYTEIHPEMRHVDCQSVWDAFKGAFISKHPCNITEEDYQPLMKLGTQTVPCNKILLWSRIKDLAHQFTQVQRDMFTLEDTLLGYLADDLTWCGEFNTSKINYQSCPDWRKDCSNNPVSVFWKTVSRRFAEAACDVVHVMLNGSRSKIFDKNSTFGSVEVHNLQPEKVQTLEAWVIHGGREDSRDLCQDPTIKELESIISKRNIQFSCKNIYRPDKFLQCVKNPEDSSCTSEI

SEQ ID NO: 12 - protein, 378 aa, homo sapiens
  CD123 antigen
MVLLWLTLLLIALPCLLQTKEDPNPPITNLRMKAKAQQLTWDLNRNVTDIECVKDADYSMPAVNNSYCQFGAISLCEVTNYTVRVANPPFSTWILFPENSGKPWAGAENLTCWIHDVDFLSCSWAVGPGAPADVQYDLYLNVANRRQQYECLHYKTDAQGTRIGCRFDDISRLSSGSQSSHILVRGRSAAFGIPCTDKFVVFSQIEILTPPNMTAKCNKTHSFMHWKMRSHFNRKFRYELQIQKRMQPVITEQVRDRTSFQLLNPGTYTVQIRARERVYEFLSAWSTPQRFECDQEEGANTRAWRTSLLIALGTLLALVCVFVICRRYLVMQRLFPRIPHMKDPIGDSFQNDKLVVWEAGKAGLEECLVTEVQVVQKT

SEQ ID NO: 13 - protein, 335 aa, homo sapiens
  CS1 antigen
MAGSPTCLTLIYILWQLTGSAASGPVKELVGSVGGAVTFPLKSKVKQVDSIVWTFNTTPLVTIQPEGGTIIVTQNRNRERVDFPDGGYSLKLSKLKKNDSGIYYVGIYSSSLQQPSTQEYVLHVYEHLSKPKVTMGLQSNKNGTCVTNLTCCMEHGEEDVIYTWKALGQAANESHNGSILPISWRWGESDMTFICVARNPVSRNFSSPILARKLCEGAADDPDSSMVLLCLLLVPLLLSLFVLGLFLWFLKRERQEEYIEEKKRVDICRETPNICPHSGENTEYDTIPHTNRTILKEDPANTVYSTVEIPKKMENPHSLLTMPDTPRLFAYENVI

SEQ ID NO: 14 - protein, 184 aa, homo sapiens
  BCMA antigen
MLQMAGQCSQNEYFDSLLHACIPCQLRCSSNTPPLTCQRYCNASVTNSVKGTNAILWTCLGLSLIISLAVFVLMFLLRKINSEPLKDEFKNTGSGLLGMANIDLEKSRTGDEIILPRGLEYTVEECTCEDCIKSKPKVDSDHCFPLPAMEEGATILVTTKTNDYCKSLPAALSATEIEKSISAR

SEQ ID NO: 15 - protein, 993 aa, homo sapiens
  FLT3 antigen
MPALARDGGQLPLLVVFSAMIFGTITNQDLPVIKCVLINHKNNDSSVGKSSSYPMVSESPEDLGCALRPQSSGTVYEAAAVEVDVSASITLQVLVDAPGNISCLWVFKHSSLNCQPHFDLQNRGVVSMVILKMTETQAGEYLLFIQSEATNYTILFTVSIRNTLLYTLRRPYFRKMENQDALVCISESVPEPIVEWVLCDSQGESCKEESPAVVKKEEKVLHELFGTDIRCCARNELGRECTRLFTIDLNQTPQTTLPQLFLKVGEPLWIRCKAVHVNHGFGLTWELENKALEEGNYFEMSTYSTNRTMIRILFAFVSSVARNDTGYYTCSSSKHPSQSALVTIVEKGFINATNSSEDYEIDQYEEFCFSVRFKAYPQIRCTWTFSRKSFPCEQKGLDNGYSISKFCNHKHQPGEYIFHAENDDAQFTKMFTLNIRRKPQVLAEASASQASCFSDGYPLPSWTWKKCSDKSPNCTEEITEGVWNRKANRKVFGQWVSSSTLNMSEAIKGFLVKCCAYNSLGTSCETILLNSPGPFPFIQDNISFYATIGVCLLFIVVLTLLICHKYKKQFRYESQLQMVQVTGSSDNEYFYVDFREYEYDLKWEFPRENLEFGKVLGSGAFGKVMNATAYGISKTGVSIQVAVKMLKEKADSSEREALMSELKMMTQLGSHENIVNLLGACTLSGPIYLIFEYCCYGDLLNYLRSKREKFHRTWTEIFKEHNFSFYPTFQSHPNSSMPGSREVQIHPDSDQISGLHGNSFHSEDEIEYENQKRLEEEEDLNVLTFEDLLCFAYQVAKGMEFLEFKSCVHRDLAARNVLVTHGKVVKICDFGLARDIMSDSNYVVRGNARLPVKWMAPESLFEGIYTIKSDVWSYGILLWEIFSLGVNPYPGIPVDANFYKLIQNGFKMDQPFYATEEIYIIMQSCWAFDSRKRPSFPNLTSFLGCQLADAEEAMYQNVDGRVSECPHTYQNRRPFSREMDLGLLSPQAQVEDS

SEQ ID NO: 16 - protein, 364 aa, homo sapiens
  CD33 antigen
MPLLLLLPLLWAGALAMDPNFWLQVQESVTVQEGLCVLVPCTFFHPIPYYDKNSPVHGYWFREGAIISRDSPVATNKLDQEVQEETQGRFRLLGDPSRNNCSLSIVDARRRDNGSYFFRMERGSTKYSYKSPQLSVHVTDLTHRPKILIPGTLEPGHSKNLTCSVSWACEQGTPPIFSWLSAAPTSLGPRTTHSSVLIITPRPQDHGTNLTCQVKFAGAGVTTERTIQLNVTYVPQNPTTGIFPGDGSGKQETRAGVVHGAIGGAGVTALLALCLCLIFFIVKTHRRKAARTAVGRNDTHPTTGSASPKHQKKSKLHGPTETSSCSGAAPTVEMDEELHYASLNFHGMNPSKDTSTEYSEVRTQ

SEQ ID NO: 17 - protein, 193 aa, homo sapiens
  CD70 antigen
MPEEGSGCSVRRRPYGCVLRAALVPLVAGLVICLVVCIQRFAQAQQQLPLESLGWDVAELQLNHTGPQQDPRLYWQGGPALGRSFLHGPELDKGQLRIHRDGIYMVHIQVTLAICSSTTASRHHPTTLAVGICSPASRSISLLRLSFHQGCTIASQRLTPLARGDTLCTNLTGTLLPSRNTDETFFGVQWVRP

SEQ ID NO: 18 - protein, 943 aa, homo sapiens
  EGFRvIII
MRPSGTAGAALLALLAALCPASRALEEKKGNYVVTDHGSCVRACGADSYEMEEDGVRKCKKCEGPCRKVCNGIGIGEFKDSLSINATNIKHFKNCTSISGDLHILPVAFRGDSFTHTPPLDPQELDILKTVKEITGFLLIQAWPENRTDLHAFENLEIIRGRTKQHGQFSLAVVSLNITSLGLRSLKEISDGDVIISGNKNLCYANTINWKKLFGTSGQKTKIISNRGENSCKATGQVCHALCSPEGCWGPEPRDCVSCRNVSRGRECVDKCNLLEGEPREFVENSECIQCHPECLPQAMNITCTGRGPDNCIQCAHYIDGPHCVKTCPAGVMGENNTLVWKYADAGHVCHLCHPNCTYGCTGPGLEGCPTNGPKIPSIATGMVGALLLLLVVALGIGLFMRRRHIVRKRTLRRLLQERELVEPLTPSGEAPNQALLRILKETEFKKIKVLGSGAFGTVYKGLWIPEGEKVKIPVAIKELREATSPKANKEILDEAYVMASVDNPHVCRLLGICLTSTVQLITQLMPFGCLLDYVREHKDNIGSQYLLNWCVQIAKGMNYLEDRRLVHRDLAARNVLVKTPQHVKITDFGLAKLLGAEEKEYHAEGGKVPIKWMALESILHRIYTHQSDVWSYGVTVWELMTFGSKPYDGIPASEISSILEKGERLPQPPICTIDVYMIMVKCWMIDADSRPKFRELIIEFSKMARDPQRYLVIQGDERMHLPSPTDSNFYRALMDEEDMDDVVDADEYLIPQQGFFSSPSTSRTPLLSSLSATSNNSTVACIDRNGLQSCPIKEDSFLQRYSSDPTGALTEDSIDDTFLPVPEYINQSVPKRPAGSVQNPVYHNQPLNPAPSRDPHYQDPHSTAVGNPEYLNTVQPTCVNSTFDSPAHWAQKGSHQISLDNPDYQQDFFPKEAKPNGIFKGSTAENAEYLRVAPQSSEFIGA

SEQ ID NO: 19 - protein, 497 aa, homo sapiens
  WT1
MQDPASTCVPEPASQHTLRSGPGCLQQPEQQGVRDPGGIWAKLGAAEASAERLQGRRSRGASGSEPQQMGSDVRDLNALLPAVPSLGGGGGCALPVSGAAQWAPVLDFAPPGASAYGSLGGPAPPPAPPPPPPPPPHSFIKQEPSWGGAEPHEEQCLSAFTVHFSGQFTGTAGACRYGPFGPPPPSQASSGQARMFPNAPYLPSCLESQPAIRNQGYSTVTFDGTPSYGHTPSHHAAQFPNHSFKHEDPMGQQGSLGEQQYSVPPPVYGCHTPTDSCTGSQALLLRTPYSSDNLYQMTSQLECMTWNQMNLGATLKGHSTGYESDNHTTPILCGAQYRIHTHGVFRGIQDVRRVPGVAPTLVRSASETSEKRPFMCAYPGCNKRYFKLSHLQMHSRKHTGEKPYQCDFKDCERRFSRSDQLKRHQRRHTGVKPFQCKTCQRKFSRSDHLKTHTRTHTGEKPFSCRWPSCQKKFARSDELVRHHNMHQRNMTKLQLAL

SEQ ID NO: 20 - DNA, 58 bp, homo sapiens
  Beta2M target 1
tctcgctccgtggccttagctgtgctcgcgctactctctctttctggcctggaggcta

SEQ ID NO: 21 - protein, 936 aa, artificial sequence
  Left Talen for beta2M target 1
MGDPKKKRKVIDYPYDVPDYAIDIADLRTLGYSQQQQEKIKPKVRSTVAQHHEALVGHGFTHAHIVALSQHPAALGTVAVKYQDMIAALPEATHEAIVGVGKQWSGARALEALLTVAGELRGPPLQLDTGQLLKIAKRGGVTAVEAVHAWRNALTGAPLNLTPQQVVAIASNNGGKQALETVQRLLPVLCQAHGLTPQQVVAIASNNGGKQALETVQRLLPVLCQAHGLTPEQVVAIASHDGGKQALETVQRLLPVLCQAHGLTPEQVVAIASHDGGKQALETVQRLLPVLCQAHGLTPQQVVAIASNGGGKQALETVQRLLPVLCQAHGLTPQQVVAIASNGGGKQALETVQRLLPVLCQAHGLTPEQVVAIASNIGGKQALETVQALLPVLCQAHGLTPQQVVAIASNNGGKQALETVQRLLPVLCQAHGLTPEQVVAIASHDGGKQALETVQRLLPVLCQAHGLTPQQVVAIASNGGGKQALETVQRLLPVLCQAHGLTPQQVVAIASNNGGKQALETVQRLLPVLCQAHGLTPQQVVAIASNGGGKQALETVQRLLPVLCQAHGLTPQQVVAIASNNGGKQALETVQRLLPVLCQAHGLTPEQVVAIASHDGGKQALETVQRLLPVLCQAHGLTPQQVVAIASNGGGKQALETVQRLLPVLCQAHGLTPQQVVAIASNGGGRPALESIVAQLSRPDPALAALTNDHLVALACLGGRPALDAVKKGLGDPISRSQLVKSELEEKKSELRHKLKYVPHEYIELIEIARNSTQDRILEMKVMEFFMKVYGYRGKHLGGSRKPDGAIYTVGSPIDYGVIVDTKAYSGGYNLPIGQADEMQRYVEENQTRNKHINPNEWWKVYPSSVTEFKFLFVSGHFKGNYKAQLTRLNHITNCNGAVLSVEELLIGGEMIKAGTLTLEEVRRKFNNGEINFAAD

SEQ ID NO: 22 - protein, 942 aa, artificial sequence
  Right Talen for beta2M target 1
MGDPKKKRKVIDKETAAAKFERQHMDSIDIADLRTLGYSQQQQEKIKPKVRSTVAQHHEALVGHGFTHAHIVALSQHPAALGTVAVKYQDMIAALPEATHEAIVGVGKQWSGARALEALLTVAGELRGPPLQLDTGQLLKIAKRGGVTAVEAVHAWRNALTGAPLNLTPEQVVAIASNIGGKQALETVQALLPVLCQAHGLTPQQVVAIASNNGGKQALETVQRLLPVLCQAHGLTPEQVVAIASHDGGKQALETVQRLLPVLCQAHGLTPEQVVAIASHDGGKQALETVQRLLPVLCQAHGLTPQQVVAIASNGGGKQALETVQRLLPVLCQAHGLTPEQVVAIASHDGGKQALETVQRLLPVLCQAHGLTPEQVVAIASHDGGKQALETVQRLLPVLCQAHGLTPEQVVAIASNIGGKQALETVQALLPVLCQAHGLTPQQVVAIASNNGGKQALETVQRLLPVLCQAHGLTPQQVVAIASNNGGKQALETVQRLLPVLCQAHGLTPEQVVAIASHDGGKQALETVQRLLPVLCQAHGLTPEQVVAIASHDGGKQALETVQRLLPVLCQAHGLTPEQVVAIASNIGGKQALETVQALLPVLCQAHGLTPQQVVAIASNNGGKQALETVQRLLPVLCQAHGLTPEQVVAIASNIGGKQALETVQALLPVLCQAHGLTPQQVVAIASNGGGRPALESIVAQLSRPDPALAALTNDHLVALACLGGRPALDAVKKGLGDPISRSQLVKSELEEKKSELRHKLKYVPHEYIELIEIARNSTQDRILEMKVMEFFMKVYGYRGKHLGGSRKPDGAIYTVGSPIDYGVIVDTKAYSGGYNLPIGQADEMQRYVEENQTRNKHINPNEWWKVYPSSVTEFKFLFVSGHFKGNYKAQLTRLNHITNCNGAVLSVEELLIGGEMIKAGTLTLEEVRRKFNNGEINFAAD

SEQ ID NO: 23 - DNA, 50 bp, homo sapiens
  Beta2M target 2
tccaaagattcaggtttactcacgtcatccagcagagaatggaaagtcaa

SEQ ID NO: 24 - protein, 936 aa, artificial sequence
  Left Talen for beta2M target 2
MGDPKKKRKVIDYPYDVPDYAIDIADLRTLGYSQQQQEKIKPKVRSTVAQHHEALVGHGFTHAHIVALSQHPAALGTVAVKYQDMIAALPEATHEAIVGVGKQWSGARALEALLTVAGELRGPPLQLDTGQLLKIAKRGGVTAVEAVHAWRNALTGAPLNLTPEQVVAIASHDGGKQALETVQRLLPVLCQAHGLTPEQVVAIASHDGGKQALETVQRLLPVLCQAHGLTPEQVVAIASNIGGKQALETVQALLPVLCQAHGLTPEQVVAIASNIGGKQALETVQALLPVLCQAHGLTPEQVVAIASNIGGKQALETVQALLPVLCQAHGLTPQQVVAIASNNGGKQALETVQRLLPVLCQAHGLTPEQVVAIASNIGGKQALETVQALLPVLCQAHGLTPQQVVAIASNGGGKQALETVQRLLPVLCQAHGLTPQQVVAIASNGGGKQALETVQRLLPVLCQAHGLTPEQVVAIASHDGGKQALETVQRLLPVLCQAHGLTPEQVVAIASNIGGKQALETVQALLPVLCQAHGLTPQQVVAIASNNGGKQALETVQRLLPVLCQAHGLTPQQVVAIASNNGGKQALETVQRLLPVLCQAHGLTPQQVVAIASNGGGKQALETVQRLLPVLCQAHGLTPQQVVAIASNGGGKQALETVQRLLPVLCQAHGLTPQQVVAIASNGGGRPALESIVAQLSRPDPALAALTNDHLVALACLGGRPALDAVKKGLGDPISRSQLVKSELEEKKSELRHKLKYVPHEYIELIEIARNSTQDRILEMKVMEFFMKVYGYRGKHLGGSRKPDGAIYTVGSPIDYGVIVDTKAYSGGYNLPIGQADEMQRYVEENQTRNKHINPNEWWKVYPSSVTEFKFLFVSGHFKGNYKAQLTRLNHITNCNGAVLSVEELLIGGEMIKAGTLTLEEVRRKFNNGEINFAAD

SEQ ID NO: 25 - protein, 942 aa, artificial sequence
  Right Talen for beta2M target 2
MGDPKKKRKVIDKETAAAKFERQHMDSIDIADLRTLGYSQQQQEKIKPKVRSTVAQHHEALVGHGFTHAHIVALSQHPAALGTVAVKYQDMIAALPEATHEAIVGVGKQWSGARALEALLTVAGELRGPPLQLDTGQLLKIAKRGGVTAVEAVHAWRNALTGAPLNLTPQQVVAIASNNGGKQALETVQRLLPVLCQAHGLTPEQVVAIASNIGGKQALETVQALLPVLCQAHGLTPEQVVAIASHDGGKQALETVQRLLPVLCQAHGLTPQQVVAIASNGGGKQALETVQRLLPVLCQAHGLTPQQVVAIASNGGGKQALETVQRLLPVLCQAHGLTPQQVVAIASNGGGKQALETVQRLLPVLCQAHGLTPEQVVAIASHDGGKQALETVQRLLPVLCQAHGLTPEQVVAIASHDGGKQALETVQRLLPVLCQAHGLTPEQVVAIASNIGGKQALETVQALLPVLCQAHGLTPQQVVAIASNGGGKQALETVQRLLPVLCQAHGLTPQQVVAIASNGGGKQALETVQRLLPVLCQAHGLTPEQVVAIASHDGGKQALETVQRLLPVLCQAHGLTPQQVVAIASNGGGKQALETVQRLLPVLCQAHGLTPEQVVAIASHDGGKQALETVQRLLPVLCQAHGLTPQQVVAIASNGGGKQALETVQRLLPVLCQAHGLTPQQVVAIASNGGGRPALESIVAQLSRPDPALAALTNDHLVALACLGGRPALDAVKKGLGDPISRSQLVKSELEEKKSELRHKLKYVPHEYIELIEIARNSTQDRILEMKVMEFFMKVYGYRGKHLGGSRKPDGAIYTVGSPIDYGVIVDTKAYSGGYNLPIGQADEMQRYVEENQTRNKHINPNEWWKVYPSSVTEFKFLFVSGHFKGNYKAQLTRLNHITNCNGAVLSVEELLIGGEMIKAGTLTLEEVRRKFNNGEINFAAD

SEQ ID NO: 26 - DNA, 47 bp, homo sapiens
  Beta2M target 3
ttagctgtgctcgcgctactctctctttctggcctggaggctatcca

SEQ ID NO: 27 - protein, 936 aa, artificial sequence
  Left Talen for beta2M target 3
MGDPKKKRKVIDYPYDVPDYAIDIADLRTLGYSQQQQEKIKPKVRSTVAQHHEALVGHGFTHAHIVALSQHPAALGTVAVKYQDMIAALPEATHEAIVGVGKQWSGARALEALLTVAGELRGPPLQLDTGQLLKIAKRGGVTAVEAVHAWRNALTGAPLNLTPEQVVAIASNIGGKQALETVQALLPVLCQAHGLTPQQVVAIASNNGGKQALETVQRLLPVLCQAHGLTPEQVVAIASHDGGKQALETVQRLLPVLCQAHGLTPQQVVAIASNGGGKQALETVQRLLPVLCQAHGLTPQQVVAIASNNGGKQALETVQRLLPVLCQAHGLTPQQVVAIASNGGGKQALETVQRLLPVLCQAHGLTPQQVVAIASNNGGKQALETVQRLLPVLCQAHGLTPEQVVAIASHDGGKQALETVQRLLPVLCQAHGLTPQQVVAIASNGGGKQALETVQRLLPVLCQAHGLTPEQVVAIASHDGGKQALETVQRLLPVLCQAHGLTPQQVVAIASNNGGKQALETVQRLLPVLCQAHGLTPEQVVAIASHDGGKQALETVQRLLPVLCQAHGLTPQQVVAIASNNGGKQALETVQRLLPVLCQAHGLTPEQVVAIASHDGGKQALETVQRLLPVLCQAHGLTPQQVVAIASNGGGKQALETVQRLLPVLCQAHGLTPQQVVAIASNGGGRPALESIVAQLSRPDPALAALTNDHLVALACLGGRPALDAVKKGLGDPISRSQLVKSELEEKKSELRHKLKYVPHEYIELIEIARNSTQDRILEMKVMEFFMKVYGYRGKHLGGSRKPDGAIYTVGSPIDYGVIVDTKAYSGGYNLPIGQADEMQRYVEENQTRNKHINPNEWWKVYPSSVTEFKFLFVSGHFKGNYKAQLTRLNHITNCNGAVLSVEELLIGGEMIKAGTLTLEEVRRKFNNGEINFAAD

SEQ ID NO: 28 - protein, 942 aa, artificial sequence
  Right Talen for beta2M target 3
MGDPKKKRKVIDKETAAAKFERQHMDSIDIADLRTLGYSQQQQEKIKPKVRSTVAQHHEALVGHGFTHAHIVALSQHPAALGTVAVKYQDMIAALPEATHEAIVGVGKQWSGARALEALLTVAGELRGPPLQLDTGQLLKIAKRGGVTAVEAVHAWRNALTGAPLNLTPQQVVAIASNNGGKQALETVQRLLPVLCQAHGLTPQQVVAIASNNGGKQALETVQRLLPVLCQAHGLTPEQVVAIASNIGGKQALETVQALLPVLCQAHGLTPQQVVAIASNGGGKQALETVQRLLPVLCQAHGLTPEQVVAIASNIGGKQALETVQALLPVLCQAHGLTPQQVVAIASNNGGKQALETVQRLLPVLCQAHGLTPEQVVAIASHDGGKQALETVQRLLPVLCQAHGLTPEQVVAIASHDGGKQALETVQRLLPVLCQAHGLTPQQVVAIASNGGGKQALETVQRLLPVLCQAHGLTPEQVVAIASHDGGKQALETVQRLLPVLCQAHGLTPEQVVAIASHDGGKQALETVQRLLPVLCQAHGLTPEQVVAIASNIGGKQALETVQALLPVLCQAHGLTPQQVVAIASNNGGKQALETVQRLLPVLCQAHGLTPQQVVAIASNNGGKQALETVQRLLPVLCQAHGLTPEQVVAIASHDGGKQALETVQRLLPVLCQAHGLTPQQVVAIASNGGGRPALESIVAQLSRPDPALAALTNDHLVALACLGGRPALDAVKKGLGDPISRSQLVKSELEEKKSELRHKLKYVPHEYIELIEIARNSTQDRILEMKVMEFFMKVYGYRGKHLGGSRKPDGAIYTVGSPIDYGVIVDTKAYSGGYNLPIGQADEMQRYVEENQTRNKHINPNEWWKVYPSSVTEFKFLFVSGHFKGNYKAQLTRLNHITNCNGAVLSVEELLIGGEMIKAGTLTLEEVRRKFNNGEINFAAD

SEQ ID NO: 29 - protein, 119 aa, homo sapiens
  &#946;2m protein sequence
MSRSVALAVLALLSLSGLEAIQRTPKIQVYSRHPAENGKSNFLNCYVSGFHPSDIEVDLLKNGERIEKVEHSDLSFSKDWSFYLLYYTEFTPTEKDEYACRVNHVTLSQPKIVKWDRDM

SEQ ID NO: 30 - protein, 238 aa, Jellyfish
  GFP protein
MSKGEELFTGVVPILVELDGDVNGHKFSVSGEGEGDATYGKLTLKFICTTGKLPVPWPTLVTTFSYGVQCFSRYPDHMKQHDFFKSAMPEGYVQERTIFFKDDGNYKTRAEVKFEGDTLVNRIELKGIDFKEDGNILGHKLEYNYNSHNVYIMADKQKNGIKVNFKIRHNIEDGSVQLADHYQQNTPIGDGPVLLPDNHYLSTQSALSKDPNEKRDHMVLLEFVTAAGITHGMDELYK